European Patent Application EP 4 806 995 A1, published September 16, 2026. Title: CRISPR-Cas系统及其应用. Applicant: 微光基因（苏州）有限公司. Application CN 202311464815.0, filed November 6, 2023. The sequence listing filed with the application follows.

SEQUENCE LISTING (97 sequences)

SEQ ID NO: 1 - protein, 1044 aa, synthetic construct
MSSAIKSYKSVLRPNERKNQLLKSTIQCLEDGSAFFFKMLQGLFGGITPEIVRFSTEQEKQQQDIALWCAVNWFRPVSQDSLTHTIASDNLVEKFEEYYGGTASDAIKQYFSASIGESYYWNDCRQQYYDLCRELGVEVSDLTHDLEILCREKCLAVATESNQYNSIISVLFGTGRKEDRSVKLRITKKILEAISNLKEIPKNVAPIQEIILNVAKATKETFRQVYAGNLGAPSTLERFIAKDGQKEFDLKKLQTDLKKVIRGKSKERDWCCQEELRSYVEQNTIQYDLWAWGEMFNKAHTALKIKSTRNYNFAKQRLEQFKRIQSLNNLLVVKKLNDFFDSEFFSGEETYTICVHHLGGKRLSKLYKAWEDDPADPENAIVVLCDDLKNNFKKEPIRNILRYIFTIRQECSAQDILAAAKYNQQLDRYKSQKANPSVLGNQGFTWRNAVILPEKAQRNDRPNSLDLRIWLYLKLRHPDGRWKKHHIPFYDTRFFQEIYAAGNSPVDTCQFRTPRFGYHLPKLTDQTAIRVNKKHVKAAKTEARIRLAIQQGTLPVSNLKITRISATINSKGQVRIPVKFDVGRQKGTLQIGDRFCGYDQNQTASHAYSLWEVVKEGQYHKELGCFVRFISSGDIVSITENRGNQFDQLSYEGLAYPQYADWRKKASKFVSLWQITKKNKKKEIVTVEAKEKFDAICKYQPRLYKFNKEYAYLLRDIVRGKSLVELQQIRQEIFRFIEQDCGVTRLGSLSLSTLETVKAVKGIIYSYFSTALNASKNNPISDEQRKEFDPELFALLEKLELIRTRKKKQKVERIANSLIQTCLENNIKFIRGEGDLSTTNNATKKKANSRSMDWLARGVFNKIRQLAPMHNITLFGCGSLYTSHQDPLVHRNPDKAMRARFEEVNVENIAEWHVRNFSNYLRADSGTGLYYKQATMDFLKHYGLEEHAEGLENKKIKFYDFRKILEDKNLTSVIIPKRGGRIYMATNPVTSDSTPITYAGKTYNRCNADHVAAANIALTVKGIGEQSSDEENPDGSRIKLQLTS

SEQ ID NO: 2 - protein, 1044 aa, synthetic construct
MSSAIKSYKSVLRPNERKNQLLKSTIQCLEDGSAFFFKMLQGLFGGITPEIVRFSTEQEKQQQDIALWCAVNWFRPVSQDSLTHTIASDNLVEKFEEYYGGTASDAIKQYFSASIGESYYWNDCRQQYYDLCRELGVEVSDLTHDLEILCREKCLAVATESNQYNSIISVLFGTGRKEDRSVKLRITKKILEAISNLKEIPKNVAPIQEIILNVAKATKETFRQVYAGNLGAPSTLERFIAKDGQKEFDLKKLQTDLKKVIRGKSKERDWCCQEELRSYVEQNTIQYDLWAWGEMFNKAHTALKIKSTRNYNFAKQRLEQFKRIQSLNNLLVVKKLNDFFDSEFFSGEETYTICVHHLGGKRLSKLYKAWEDDPADPENAIVVLCDDLKNNFKKEPIRNILRYIFTIRQECSAQDILAAAKYNQQLDRYKSQKANPSVLGNQGFTWRNAVILPEKAQRNDRPNSLDLRIWLYLKLRHPDGRWKKHHIPFYDTRFFQEIYAAGNSPVDTCQFRTPRFGYHLPKLTDQTAIRVNKKHVKAAKTEARIRLAIQQGTLPVSNLKITRISATINSKGQVRIPVKFDVGRQKGTLQIGDRFCGYDQNQTASHAYSLWEVVKEGQYHKELGCFVRFISSGDIVSITENRGNQFDQLSYEGLAYPQYADWRKKASKFVSLWQITKKNKKKEIVTVEAKEKFDAICKYQPRLYKFNKEYAYLLRDIVRGKSLVELQQIRQEIFRFIEQDCGVTRLGSLSLSTLETVKAVKGIIYSYFSTALNASKNNPISDEQRKEFDPELFALLEKLELIRTRKKKQKVERIANSLIQTCLENNIKFIRGEGDLSTTNNATKKKANSRSMDWLARGVFNKIRQLAPMHNITLFGCGSLYTSHQDPLVHRNPDKAMRARFEEVNVSNVSEWHMRNFSNYLRADSGTGLYYKQATLDFLKHYDLEEHADDLEKQNIKFYDFRKILEDKQLTSVIVPKRGGRIYMATNPVTSDSTPVTYAGKTYNRCNADHVAAANIALTVKGIGEQSSDEENPDGSRIKLQLTS

SEQ ID NO: 3 - protein, 1054 aa, synthetic construct
MSSAIKSYKSVLRPNERKNQLLKSTIQCLEDGSAFFFKMLQGLFGGITPEIVRFSTEQEKQQQDIALWCAVNWFRPVSQDSLTHTIASDNLVEKFEEYYGGTASDAIKQYFSASIGESYYWNDCRQQYYDLCRELGVEVSDLTHDLEILCREKCLAVATESNQYNSIISVLFGTGRKEDRSVKLRITKKILEAISNLKEIPKNVAPIQEIILNVAKATKETFRQVYAGNLGAPSTLERFIAKDGQKEFDLKKLQTDLKKVIRGKSKERDWCCQEELRSYVEQNTIQYDLWAWGEMFNKAHTALKIKSTRNYNFAKQRLEQFKRIQSLNNLLVVKKLNDFFDSEFFSGEETYTICVHHLGGKRLSKLYKAWEDDPADPENAIVVLCDDLKNNFKKEPIRNILRYIFTIRQECSAQDILAAAKYNQQLDRYKSQKANPSVLGNQGFTWRNAVILPEKAQRNDRPNSLDLRIWLYLKLRHPDGRWKKHHIPFYDTRFFQEIYAAGNSPVDTCQFRTPRFGYHLPKLTDQTAIRVNKKHVKAAKTEARIRLAIQQGTLPVSNLKITRISATINSKGQVRIPVKFDVGRQKGTLQIGDRFCGYDQNQTASHAYSLWEVVKEGQYHKELGCFVRFISSGDIVSITENRGNQFDQLSYEGLAYPQYADWRKKASKFVSLWQITKKNKKKEIVTVEAKEKFDAICKYQPRLYKFNKEYAYLLRDIVRGKSLVELQQIRQEIFRFIEQDCGVTRLGSLSLSTLETVKAVKGIIYSYFSTALNASKNNPISDEQRKEFDPELFALLEKLELIRTRKKKQKVERIANSLIQTCLENNIKFIRGEGDLSTTNNATKKKANSRSMDWLARGVFNKIRQLAPMHNITLFGCGSLYTSHQDPLVHRNPDKSFRARWDLVKVKDFGEKHLLTLSRNLTGKGPGTRKYYHQGVEDFLKEYELEDLKEELAKIKKGDPNALPPEVIRNKLKEKLGNENAPVLIPKRGGKYFLSTHNVATGAVKITFNNKERYLCNADHVAAANIALTVKGIGEQSSDEENPDGSRIKLQLTS

SEQ ID NO: 4 - protein, 1054 aa, synthetic construct
MSSAIKSYKSVLRPNERKNQLLKSTIQCLEDGSAFFFKMLQGLFGGITPEIVRFSTEQEKQQQDIALWCAVNWFRPVSQDSLTHTIASDNLVEKFEEYYGGTASDAIKQYFSASIGESYYWNDCRQQYYDLCRELGVEVSDLTHDLEILCREKCLAVATESNQYNSIISVLFGTGRKEDRSVKLRITKKILEAISNLKEIPKNVAPIQEIILNVAKATKETFRQVYAGNLGAPSTLERFIAKDGQKEFDLKKLQTDLKKVIRGKSKERDWCCQEELRSYVEQNTIQYDLWAWGEMFNKAHTALKIKSTRNYNFAKQRLEQFKRIQSLNNLLVVKKLNDFFDSEFFSGEETYTICVHHLGGKRLSKLYKAWEDDPADPENAIVVLCDDLKNNFKKEPIRNILRYIFTIRQECSAQDILAAAKYNQQLDRYKSQKANPSVLGNQGFTWRNAVILPEKAQRNDRPNSLDLRIWLYLKLRHPDGRWKKHHIPFYDTRFFQEIYAAGNSPVDTCQFRTPRFGYHLPKLTDQTAIRVNKKHVKAAKTEARIRLAIQQGTLPVSNLKITRISATINSKGQVRIPVKFDVGRQKGTLQIGDRFCGYDQNQTASHAYSLWEVVKEGQYHKELGCFVRFISSGDIVSITENRGNQFDQLSYEGLAYPQYADWRKKASKFVSLWQITKKNKKKEIVTVEAKEKFDAICKYQPRLYKFNKEYAYLLRDIVRGKSLVELQQIRQEIFRFIEQDCGVTRLGSLSLSTLETVKAVKGIIYSYFSTALNASKNNPISDEQRKEFDPELFALLEKLELIRTRKKKQKVERIANSLIQTCLENNIKFIRGEGDLSTTNNATKKKANSRSMDWLARGVFNKIRQLAPMHNITLFGCGSLYTSHQDPLVHRNPDKSFRARWRLVKVKDIGEKELLTLSRNLRGKGKGIKKYYHQGVLDFFKEYELEELAGPLAKIKPGDPNAIPPEVLRNKLKEKLGNEDAPVLIPVAGGGIYLSTHNVATGAKKITFNNKERYVCNADHVAAANIALTVKGIGEQSSDEENPDGSRIKLQLTS

SEQ ID NO: 5 - protein, 1054 aa, synthetic construct
MSSAIKSYKSVLRPNERKNQLLKSTIQCLEDGSAFFFKMLQGLFGGITPEIVRFSTEQEKQQQDIALWCAVNWFRPVSQDSLTHTIASDNLVEKFEEYYGGTASDAIKQYFSASIGESYYWNDCRQQYYDLCRELGVEVSDLTHDLEILCREKCLAVATESNQYNSIISVLFGTGRKEDRSVKLRITKKILEAISNLKEIPKNVAPIQEIILNVAKATKETFRQVYAGNLGAPSTLERFIAKDGQKEFDLKKLQTDLKKVIRGKSKERDWCCQEELRSYVEQNTIQYDLWAWGEMFNKAHTALKIKSTRNYNFAKQRLEQFKRIQSLNNLLVVKKLNDFFDSEFFSGEETYTICVHHLGGKRLSKLYKAWEDDPADPENAIVVLCDDLKNNFKKEPIRNILRYIFTIRQECSAQDILAAAKYNQQLDRYKSQKANPSVLGNQGFTWRNAVILPEKAQRNDRPNSLDLRIWLYLKLRHPDGRWKKHHIPFYDTRFFQEIYAAGNSPVDTCQFRTPRFGYHLPKLTDQTAIRVNKKHVKAAKTEARIRLAIQQGTLPVSNLKITRISATINSKGQVRIPVKFDVGRQKGTLQIGDRFCGYDQNQTASHAYSLWEVVKEGQYHKELGCFVRFISSGDIVSITENRGNQFDQLSYEGLAYPQYADWRKKASKFVSLWQITKKNKKKEIVTVEAKEKFDAICKYQPRLYKFNKEYAYLLRDIVRGKSLVELQQIRQEIFRFIEQDCGVTRLGSLSLSTLETVKAVKGIIYSYFSTALNASKNNPISDEQRKEFDPELFALLEKLELIRTRKKKQKVERIANSLIQTCLENNIKFIRGEGDLSTTNNATKKKANSRSMDWLARGVFNKIRQLAPMHNITLFGCGSLYTSHQDPLVHRNPDKKYNARWDLVKVKDIGEGHLLILSRNLRGKGSGIRKYYHQGVLEFFKEYDLEDLAEPLAKIRPGDPNAIPPEVLRERLKEKLGNEDAPVLIPKPGGGVYLSTHNVATGAKKITFNNKERYLCNADHVAAANIALTVKGIGEQSSDEENPDGSRIKLQLTS

SEQ ID NO: 6 - protein, 1054 aa, synthetic construct
MSSAIKSYKSVLRPNERKNQLLKSTIQCLEDGSAFFFKMLQGLFGGITPEIVRFSTEQEKQQQDIALWCAVNWFRPVSQDSLTHTIASDNLVEKFEEYYGGTASDAIKQYFSASIGESYYWNDCRQQYYDLCRELGVEVSDLTHDLEILCREKCLAVATESNQYNSIISVLFGTGRKEDRSVKLRITKKILEAISNLKEIPKNVAPIQEIILNVAKATKETFRQVYAGNLGAPSTLERFIAKDGQKEFDLKKLQTDLKKVIRGKSKERDWCCQEELRSYVEQNTIQYDLWAWGEMFNKAHTALKIKSTRNYNFAKQRLEQFKRIQSLNNLLVVKKLNDFFDSEFFSGEETYTICVHHLGGKRLSKLYKAWEDDPADPENAIVVLCDDLKNNFKKEPIRNILRYIFTIRQECSAQDILAAAKYNQQLDRYKSQKANPSVLGNQGFTWRNAVILPEKAQRNDRPNSLDLRIWLYLKLRHPDGRWKKHHIPFYDTRFFQEIYAAGNSPVDTCQFRTPRFGYHLPKLTDQTAIRVNKKHVKAAKTEARIRLAIQQGTLPVSNLKITRISATINSKGQVRIPVKFDVGRQKGTLQIGDRFCGYDQNQTASHAYSLWEVVKEGQYHKELGCFVRFISSGDIVSITENRGNQFDQLSYEGLAYPQYADWRKKASKFVSLWQITKKNKKKEIVTVEAKEKFDAICKYQPRLYKFNKEYAYLLRDIVRGKSLVELQQIRQEIFRFIEQDCGVTRLGSLSLSTLETVKAVKGIIYSYFSTALNASKNNPISDEQRKEFDPELFALLEKLELIRTRKKKQKVERIANSLIQTCLENNIKFIRGEGDLSTTNNATKKKANSRSMDWLARGVFNKIRQLAPMHNITLFGCGSLYTSHQDPLVHRNPDKSYRARWRLVRVRDFGERHLLTLSRNLTGKGKGTRKYYHQGVLDFFREYDLEDLAGPLAKIRPGDPDAIPPEVLRERLREKLGNDEAPVLIPVRGGPVYLSTHDVATGAKRITFNGKERYLCNADHVAAANIALTVKGIGEQSSDEENPDGSRIKLQLTS

SEQ ID NO: 7 - RNA, 23 nt, synthetic construct
  source 1..23: mol_type = other RNA
agaaatccgtctttcattgacgg

SEQ ID NO: 8 - RNA, 23 nt, synthetic construct
  source 1..23: mol_type = other RNA
agaaatgtgtccccagttgacac

SEQ ID NO: 9 - RNA, 23 nt, synthetic construct
  source 1..23: mol_type = other RNA
agaaatccgtccttagttgacgg

SEQ ID NO: 10 - RNA, 22 nt, synthetic construct
  source 1..22: mol_type = other RNA
agacatgtgtccccagtgacac

SEQ ID NO: 11 - RNA, 23 nt, synthetic construct
  source 1..23: mol_type = other RNA
agaaatgtttccccagttgaaac

SEQ ID NO: 12 - RNA, 23 nt, synthetic construct
  source 1..23: mol_type = other RNA
agaaatgtgttcccagttaacac

SEQ ID NO: 13 - RNA, 23 nt, synthetic construct
  source 1..23: mol_type = other RNA
agaaatttgtccccagttgacaa

SEQ ID NO: 14 - RNA, 23 nt, synthetic construct
  source 1..23: mol_type = other RNA
agaaatccgtcctacgttgacgg

SEQ ID NO: 15 - RNA, 24 nt, synthetic construct
  source 1..24: mol_type = other RNA
nagaaatccgtctttcattgacgg

SEQ ID NO: 16 - RNA, 24 nt, synthetic construct
  source 1..24: mol_type = other RNA
nagaaatgtgtccccagttgacac

SEQ ID NO: 17 - RNA, 24 nt, synthetic construct
  source 1..24: mol_type = other RNA
nagaaatccgtccttagttgacgg

SEQ ID NO: 18 - RNA, 23 nt, synthetic construct
  source 1..23: mol_type = other RNA
nagacatgtgtccccagtgacac

SEQ ID NO: 19 - RNA, 24 nt, synthetic construct
  source 1..24: mol_type = other RNA
nagaaatgtttccccagttgaaac

SEQ ID NO: 20 - RNA, 24 nt, synthetic construct
  source 1..24: mol_type = other RNA
nagaaatgtgttcccagttaacac

SEQ ID NO: 21 - RNA, 24 nt, synthetic construct
  source 1..24: mol_type = other RNA
nagaaatttgtccccagttgacaa

SEQ ID NO: 22 - RNA, 24 nt, synthetic construct
  source 1..24: mol_type = other RNA
nagaaatccgtcctacgttgacgg

SEQ ID NO: 23 - protein, 167 aa, synthetic construct
MSEVEFSHEYWMRHALTLAKRAWDEREVPVGAVLVHNNRVIGEGWNRPIGRHDPTAHAEIMALRQGGLVMQNYRLIDATLYVTLEPCVMCAGAMIHSRIGRVVFGARDAKTGAAGSLMDVLHHPGMNHRVEITEGILADECAALLSDFFRMRRQEIKAQKKAQSSTD

SEQ ID NO: 24 - protein, 178 aa, synthetic construct
MRRAFITGVFFLSEVEFSHEYWMRHALTLAKRAWDEREVPVGAVLVHNNRVIGEGWNRPIGRHDPTAHAEIMALRQGGLVMQNYRLIDATLYVTLEPCVMCAGAMIHSRIGRVVFGARDAKTGAAGSLMDVLHHPGMNHRVEITEGILADECAALLSDFFRMRRQEIKAQKKAQSSTD

SEQ ID NO: 25 - protein, 160 aa, synthetic construct
MGSHMTNDIYFMTLAIEEAKKAAQLGEVPIGAIITKDDEVIARAHNLRETLQQPTAHAEHIAIERAAKVLGSWRLEGCTLYVTLEPCVMCAGTIVMSRIPRVVYGADDPKGGCSGSLMNLLQQSNFNHRAIVDKGVLKEACSTLLTTFFKNLRANKKSTN

SEQ ID NO: 26 - protein, 161 aa, synthetic construct
MTQDELYMKEAIKEAKKAEEKGEVPIGAVLVINGEIIARAHNLRETEQRSIAHAEMLVIDEACKALGTWRLEGATLYVTLEPCPMCAGAVVLSRVEKVVFGAFDPKGGCSGTLMNLLQEERFNHQAEVVSGVLEEECGGMLSAFFRELRKKKKAARKNLSE

SEQ ID NO: 27 - protein, 183 aa, synthetic construct
MPPAFITGVTSLSDVELDHEYWMRHALTLAKRAWDEREVPVGAVLVHNHRVIGEGWNRPIGRHDPTAHAEIMALRQGGLVLQNYRLLDTTLYVTLEPCVMCAGAMVHSRIGRVVFGARDAKTGAAGSLIDVLHHPGMNHRVEIIEGVLRDECATLLSDFFRMRRQEIKALKKADRAEGAGPAV

SEQ ID NO: 28 - protein, 164 aa, synthetic construct
MDEYWMQVAMQMAEKAEAAGEVPVGAVLVKDGQQIATGYNLSISQHDPTAHAEILCLRSAGKKLENYRLLDATLYITLEPCAMCAGAMVHSRIARVVYGARDEKTGAAGTVVNLLQHPAFNHQVEVTSGVLAEACSAQLSRFFKRRRDEKKALKLAQRAQQGIE

SEQ ID NO: 29 - protein, 173 aa, synthetic construct
MDAAKVRSEFDEKMMRYALELADKAEALGEIPVGAVLVDDARNIIGEGWNLSIVQSDPTAHAEIIALRNGAKNIQNYRLLNSTLYVTLEPCTMCAGAILHSRIKRLVFGASDYKTGAIGSRFHFFDDYKMNHTLEITSGVLAEECSQKLSTFFQKRREEKKIEKALLKSLSDK

SEQ ID NO: 30 - protein, 161 aa, synthetic construct
MRTDESEDQDHRMMRLALDAARAAAEAGETPVGAVILDPSTGEVIATAGNGPIAAHDPTAHAEIAAMRAAAAKLGNYRLTDLTLVVTLEPCAMCAGAISHARIGRVVFGADDPKGGAVVHGPKFFAQPTCHWRPEVTGGVLADESADLLRGFFRARRKAKI

SEQ ID NO: 31 - protein, 179 aa, synthetic construct
MSSLKKTPIRDDAYWMGKAIREAAKAAARDEVPIGAVIVRDGAVIGRGHNLREGSNDPSAHAEMIAIRQAARRSANWRLTGATLYVTLEPCLMCMGAIILARLERVVFGCYDPKGGAAGSLYDLSADPRLNHQVRLSPGVCQEECGTMLSDFFRDLRRRKKAKATPALFIDERKVPPEP

SEQ ID NO: 32 - protein, 198 aa, synthetic construct [sequence omitted]

SEQ ID NO: 33 - protein, 188 aa, synthetic construct
MDSLLMNRRKFLYQFKNVRWAKGRRETYLCYVVKRRDSATSFSLDFGYLRNKNGCHVELLFLRYISDWDLDPGRCYRVTWFTSWSPCYDCARHVADFLRGNPNLSLRIFTARLYFCEDRKAEPEGLRRLHRAGVQIAIMTFKENHERTFKAWEGLHENSVRLSRQLRRILLPLYEVDDLRDAFRTLGL

SEQ ID NO: 34 - protein, 198 aa, synthetic construct [sequence omitted]

SEQ ID NO: 35 - protein, 7 aa, synthetic construct
PKKKRKV

SEQ ID NO: 36 - protein, 16 aa, synthetic construct
KRPAATKKAGQAKKKK

SEQ ID NO: 37 - protein, 9 aa, synthetic construct
PAAKRVKLD

SEQ ID NO: 38 - protein, 11 aa, synthetic construct
RQRRNELKRSP

SEQ ID NO: 39 - protein, 38 aa, synthetic construct
NQSSNFGPMKGGNFGGRSSGPYGGGGQYFAKPRNQGGY

SEQ ID NO: 40 - protein, 42 aa, synthetic construct
RMRIZFKNKGKDTAELRRRRVEVSVELRKAKKDEQILKRRNV

SEQ ID NO: 41 - protein, 8 aa, synthetic construct
VSRKRPRP

SEQ ID NO: 42 - protein, 8 aa, synthetic construct
PPKKARED

SEQ ID NO: 43 - protein, 8 aa, synthetic construct
PQPKKKPL

SEQ ID NO: 44 - protein, 12 aa, synthetic construct
SALIKKKKKMAP

SEQ ID NO: 45 - protein, 5 aa, synthetic construct
DRLRR

SEQ ID NO: 46 - protein, 7 aa, synthetic construct
PKQKKRK

SEQ ID NO: 47 - protein, 10 aa, synthetic construct
RKLKKKIKKL

SEQ ID NO: 48 - protein, 10 aa, synthetic construct
REKKKFLKRR

SEQ ID NO: 49 - protein, 20 aa, synthetic construct
KRKGDEVDGVDEVAKKKSKK

SEQ ID NO: 50 - protein, 17 aa, synthetic construct
RKCLQAGMNLEARKTKK

SEQ ID NO: 51 - protein, 5 aa, synthetic construct
GGSGG

SEQ ID NO: 52 - protein, 5 aa, synthetic construct
GSGSG

SEQ ID NO: 53 - protein, 5 aa, synthetic construct
GSGGG

SEQ ID NO: 54 - protein, 5 aa, synthetic construct
GGGSG

SEQ ID NO: 55 - protein, 5 aa, synthetic construct
GSSSG

SEQ ID NO: 56 - protein, 8 aa, synthetic construct
SGGSSGGS

SEQ ID NO: 57 - protein, 16 aa, synthetic construct
SGSETPGTSESATPES

SEQ ID NO: 58 - protein, 24 aa, synthetic construct
SGGSSGSETPGTSESATPESSGGS

SEQ ID NO: 59 - DNA, 3132 bp, synthetic construct
  source 1..3132: mol_type = other DNA
atgagcagcgccatcaagagctacaagagcgtgctgcgccccaacgagcgcaagaaccagctgctgaagagcaccatccagtgcctggaggacggcagcgccttcttcttcaagatgctgcagggcctgttcggcggcatcacccccgagatcgtgcgcttcagcaccgagcaggagaagcagcagcaggacatcgccctgtggtgcgccgtgaactggttccgccccgtgagccaggacagcctgacccacaccatcgccagcgacaacctggtggagaagttcgaggagtactacggcggcaccgccagcgacgccatcaagcagtacttcagcgccagcatcggcgagagctactactggaacgactgccgccagcagtactacgacctgtgccgcgagctgggcgtggaggtgagcgacctgacccacgacctggagatcctgtgccgcgagaagtgcctggccgtggccaccgagagcaaccagtacaacagcatcatcagcgtgctgttcggcaccggcagaaaggaggaccgcagcgtgaagctgcgcatcaccaagaagatcctggaggccatcagcaacctgaaggagatccccaagaacgtggcccccatccaggagatcatcctgaacgtggccaaggccaccaaggagaccttccgccaggtgtacgccggcaacctgggcgcccccagcaccctggagagattcatcgccaaggacggccagaaggagttcgacctgaagaagctgcagaccgacctgaagaaggtgatccgcggcaagagcaaggagcgcgactggtgctgccaggaggagctgcgcagctacgtggagcagaacaccatccagtacgacctgtgggcctggggcgagatgttcaacaaggcccacaccgccctgaagatcaagagcacccgcaactacaacttcgccaagcagcgcctggagcagttcaagagaatccagagcctgaacaacctgctggtggtgaagaagctgaacgacttcttcgacagcgagttcttcagcggcgaggagacctacaccatctgcgtgcaccacctgggcggcaagagactgagcaagctgtacaaggcctgggaggacgaccccgccgaccccgagaacgccatcgtggtgctgtgcgacgacctgaagaacaacttcaagaaggagcccatccgcaacatcctgcgctacatcttcaccatccgccaggagtgcagcgcccaggacatcctggccgccgccaagtacaaccagcagctggaccgctacaagagccagaaggccaaccccagcgtgctgggcaaccagggcttcacctggagaaacgccgtgatcctgcccgagaaggcccagcgcaacgaccgccccaacagcctggacctgcgcatctggctgtacctgaagctgcgccaccccgacggccgctggaagaagcaccacatccccttctacgacacccgcttcttccaggagatctacgccgccggcaacagccccgtggacacctgccagttccgcaccccccgcttcggctaccacctgcccaagctgaccgaccagaccgccatccgcgtgaacaagaagcacgtgaaggccgccaagaccgaggcccgcatccgcctggccatccagcagggcaccctgcccgtgagcaacctgaagatcaccagaatcagcgccaccatcaacagcaagggccaggtgcgcatccccgtgaagttcgacgtgggccgccagaagggcaccctgcagatcggcgaccgcttctgcggctacgaccagaaccagaccgccagccacgcctacagcctgtgggaggtggtgaaggagggccagtaccacaaggagctgggctgcttcgtgcgcttcatcagcagcggcgacatcgtgagcatcaccgagaaccgcggcaaccagttcgaccagctgagctacgagggcctggcctacccccagtacgccgactggcgcaagaaggccagcaagttcgtgagcctgtggcagatcaccaagaagaacaagaagaaggagatcgtgaccgtggaggccaaggagaagttcgacgccatctgcaagtaccagccccgcctgtacaagttcaacaaggagtacgcctacctgctgcgcgacatcgtgcgcggcaagagcctggtggagctgcagcagatccgccaggagatcttccgcttcatcgagcaggactgcggcgtgacccgcctgggcagcctgagcctgagcaccctggagaccgtgaaggccgtgaagggcatcatctacagctacttcagcaccgccctgaacgccagcaagaacaaccccatcagcgacgagcagcgcaaggagttcgaccccgagctgttcgccctgctggagaagctggagctgatccgcacccgcaagaagaagcagaaggtggagcgcatcgccaacagcctgatccagacctgcctggagaacaacatcaagttcatccgcggcgagggcgacctgagcaccaccaacaacgccaccaagaagaaggccaacagccgcagcatggactggctggcccgcggcgtgttcaacaagatccgccagctggcccccatgcacaacatcaccctgttcggctgcggcagcctgtacaccagccaccaggaccccctggtgcaccgcaaccccgacaaggccatgagggcaaggttcgaggaggtcaacgtggagaatatcgccgagtggcatgttagaaacttctcaaattatctccgcgctgacagcgggacaggcctctattacaagcaggcaaccatggactttctgaagcactatggactggaggagcacgcagaggggctggaaaataagaaaatcaagttctatgactttcggaagattctggaagataaaaatctgaccagcgtaatcatacccaagcgaggggggcgcatctatatggccaccaacccagtaacctccgactcaacaccgataacctacgccgggaaaacatacaatagatgcaacgccgatcacgtggccgccgccaacatcgccctgaccgtgaagggcatcggcgagcagagcagcgacgaggagaaccccgacggcagccgcatcaagctgcagctgaccagc

SEQ ID NO: 60 - DNA, 3132 bp, synthetic construct
  source 1..3132: mol_type = other DNA
atgagcagcgccatcaagagctacaagagcgtgctgcgccccaacgagcgcaagaaccagctgctgaagagcaccatccagtgcctggaggacggcagcgccttcttcttcaagatgctgcagggcctgttcggcggcatcacccccgagatcgtgcgcttcagcaccgagcaggagaagcagcagcaggacatcgccctgtggtgcgccgtgaactggttccgccccgtgagccaggacagcctgacccacaccatcgccagcgacaacctggtggagaagttcgaggagtactacggcggcaccgccagcgacgccatcaagcagtacttcagcgccagcatcggcgagagctactactggaacgactgccgccagcagtactacgacctgtgccgcgagctgggcgtggaggtgagcgacctgacccacgacctggagatcctgtgccgcgagaagtgcctggccgtggccaccgagagcaaccagtacaacagcatcatcagcgtgctgttcggcaccggcagaaaggaggaccgcagcgtgaagctgcgcatcaccaagaagatcctggaggccatcagcaacctgaaggagatccccaagaacgtggcccccatccaggagatcatcctgaacgtggccaaggccaccaaggagaccttccgccaggtgtacgccggcaacctgggcgcccccagcaccctggagagattcatcgccaaggacggccagaaggagttcgacctgaagaagctgcagaccgacctgaagaaggtgatccgcggcaagagcaaggagcgcgactggtgctgccaggaggagctgcgcagctacgtggagcagaacaccatccagtacgacctgtgggcctggggcgagatgttcaacaaggcccacaccgccctgaagatcaagagcacccgcaactacaacttcgccaagcagcgcctggagcagttcaagagaatccagagcctgaacaacctgctggtggtgaagaagctgaacgacttcttcgacagcgagttcttcagcggcgaggagacctacaccatctgcgtgcaccacctgggcggcaagagactgagcaagctgtacaaggcctgggaggacgaccccgccgaccccgagaacgccatcgtggtgctgtgcgacgacctgaagaacaacttcaagaaggagcccatccgcaacatcctgcgctacatcttcaccatccgccaggagtgcagcgcccaggacatcctggccgccgccaagtacaaccagcagctggaccgctacaagagccagaaggccaaccccagcgtgctgggcaaccagggcttcacctggagaaacgccgtgatcctgcccgagaaggcccagcgcaacgaccgccccaacagcctggacctgcgcatctggctgtacctgaagctgcgccaccccgacggccgctggaagaagcaccacatccccttctacgacacccgcttcttccaggagatctacgccgccggcaacagccccgtggacacctgccagttccgcaccccccgcttcggctaccacctgcccaagctgaccgaccagaccgccatccgcgtgaacaagaagcacgtgaaggccgccaagaccgaggcccgcatccgcctggccatccagcagggcaccctgcccgtgagcaacctgaagatcaccagaatcagcgccaccatcaacagcaagggccaggtgcgcatccccgtgaagttcgacgtgggccgccagaagggcaccctgcagatcggcgaccgcttctgcggctacgaccagaaccagaccgccagccacgcctacagcctgtgggaggtggtgaaggagggccagtaccacaaggagctgggctgcttcgtgcgcttcatcagcagcggcgacatcgtgagcatcaccgagaaccgcggcaaccagttcgaccagctgagctacgagggcctggcctacccccagtacgccgactggcgcaagaaggccagcaagttcgtgagcctgtggcagatcaccaagaagaacaagaagaaggagatcgtgaccgtggaggccaaggagaagttcgacgccatctgcaagtaccagccccgcctgtacaagttcaacaaggagtacgcctacctgctgcgcgacatcgtgcgcggcaagagcctggtggagctgcagcagatccgccaggagatcttccgcttcatcgagcaggactgcggcgtgacccgcctgggcagcctgagcctgagcaccctggagaccgtgaaggccgtgaagggcatcatctacagctacttcagcaccgccctgaacgccagcaagaacaaccccatcagcgacgagcagcgcaaggagttcgaccccgagctgttcgccctgctggagaagctggagctgatccgcacccgcaagaagaagcagaaggtggagcgcatcgccaacagcctgatccagacctgcctggagaacaacatcaagttcatccgcggcgagggcgacctgagcaccaccaacaacgccaccaagaagaaggccaacagccgcagcatggactggctggcccgcggcgtgttcaacaagatccgccagctggcccccatgcacaacatcaccctgttcggctgcggcagcctgtacaccagccaccaggaccccctggtgcaccgcaaccccgacaaggccatgagagcccggtttgaggaagtgaatgttagcaacgtgtctgaatggcatatgagaaactttagcaattatttgagagccgatagcggcactggtttgtattacaagcaggccaccttggattttctgaagcactacgaccttgaggaacacgcagatgacttggagaaacagaacataaaattctacgatttccggaaaattttggaagataaacaactgacctccgtcatcgttccaaagcggggagggaggatctatatggccactaaccctgtgacgtccgatagtacccctgtgacctacgcaggaaagacatacaaccggtgcaatgccgatcacgtggccgccgccaacatcgccctgaccgtgaagggcatcggcgagcagagcagcgacgaggagaaccccgacggcagccgcatcaagctgcagctgaccagc

SEQ ID NO: 61 - DNA, 3162 bp, synthetic construct
  source 1..3162: mol_type = other DNA
atgagcagcgccatcaagagctacaagagcgtgctgcgccccaacgagcgcaagaaccagctgctgaagagcaccatccagtgcctggaggacggcagcgccttcttcttcaagatgctgcagggcctgttcggcggcatcacccccgagatcgtgcgcttcagcaccgagcaggagaagcagcagcaggacatcgccctgtggtgcgccgtgaactggttccgccccgtgagccaggacagcctgacccacaccatcgccagcgacaacctggtggagaagttcgaggagtactacggcggcaccgccagcgacgccatcaagcagtacttcagcgccagcatcggcgagagctactactggaacgactgccgccagcagtactacgacctgtgccgcgagctgggcgtggaggtgagcgacctgacccacgacctggagatcctgtgccgcgagaagtgcctggccgtggccaccgagagcaaccagtacaacagcatcatcagcgtgctgttcggcaccggcagaaaggaggaccgcagcgtgaagctgcgcatcaccaagaagatcctggaggccatcagcaacctgaaggagatccccaagaacgtggcccccatccaggagatcatcctgaacgtggccaaggccaccaaggagaccttccgccaggtgtacgccggcaacctgggcgcccccagcaccctggagagattcatcgccaaggacggccagaaggagttcgacctgaagaagctgcagaccgacctgaagaaggtgatccgcggcaagagcaaggagcgcgactggtgctgccaggaggagctgcgcagctacgtggagcagaacaccatccagtacgacctgtgggcctggggcgagatgttcaacaaggcccacaccgccctgaagatcaagagcacccgcaactacaacttcgccaagcagcgcctggagcagttcaagagaatccagagcctgaacaacctgctggtggtgaagaagctgaacgacttcttcgacagcgagttcttcagcggcgaggagacctacaccatctgcgtgcaccacctgggcggcaagagactgagcaagctgtacaaggcctgggaggacgaccccgccgaccccgagaacgccatcgtggtgctgtgcgacgacctgaagaacaacttcaagaaggagcccatccgcaacatcctgcgctacatcttcaccatccgccaggagtgcagcgcccaggacatcctggccgccgccaagtacaaccagcagctggaccgctacaagagccagaaggccaaccccagcgtgctgggcaaccagggcttcacctggagaaacgccgtgatcctgcccgagaaggcccagcgcaacgaccgccccaacagcctggacctgcgcatctggctgtacctgaagctgcgccaccccgacggccgctggaagaagcaccacatccccttctacgacacccgcttcttccaggagatctacgccgccggcaacagccccgtggacacctgccagttccgcaccccccgcttcggctaccacctgcccaagctgaccgaccagaccgccatccgcgtgaacaagaagcacgtgaaggccgccaagaccgaggcccgcatccgcctggccatccagcagggcaccctgcccgtgagcaacctgaagatcaccagaatcagcgccaccatcaacagcaagggccaggtgcgcatccccgtgaagttcgacgtgggccgccagaagggcaccctgcagatcggcgaccgcttctgcggctacgaccagaaccagaccgccagccacgcctacagcctgtgggaggtggtgaaggagggccagtaccacaaggagctgggctgcttcgtgcgcttcatcagcagcggcgacatcgtgagcatcaccgagaaccgcggcaaccagttcgaccagctgagctacgagggcctggcctacccccagtacgccgactggcgcaagaaggccagcaagttcgtgagcctgtggcagatcaccaagaagaacaagaagaaggagatcgtgaccgtggaggccaaggagaagttcgacgccatctgcaagtaccagccccgcctgtacaagttcaacaaggagtacgcctacctgctgcgcgacatcgtgcgcggcaagagcctggtggagctgcagcagatccgccaggagatcttccgcttcatcgagcaggactgcggcgtgacccgcctgggcagcctgagcctgagcaccctggagaccgtgaaggccgtgaagggcatcatctacagctacttcagcaccgccctgaacgccagcaagaacaaccccatcagcgacgagcagcgcaaggagttcgaccccgagctgttcgccctgctggagaagctggagctgatccgcacccgcaagaagaagcagaaggtggagcgcatcgccaacagcctgatccagacctgcctggagaacaacatcaagttcatccgcggcgagggcgacctgagcaccaccaacaacgccaccaagaagaaggccaacagccgcagcatggactggctggcccgcggcgtgttcaacaagatccgccagctggcccccatgcacaacatcaccctgttcggctgcggcagcctgtacaccagccaccaggaccccctggtgcaccgcaaccccgacaagtcttttagagctagatgggacctggtgaaggttaaggattttggagagaaacatctcctcacactgagcaggaatctgactggaaagggaccaggcacccgcaagtactaccaccagggagttgaggactttctgaaggagtatgagctggaggacctgaaggaagagctggccaagattaagaaaggcgacccaaacgccctccctcctgaggtgataagaaataaactgaaagaaaagctgggaaacgagaacgcaccagttctgatacctaagcgcggtggaaagtactttctgtcaacccataacgtggcaactggcgcagtgaaaatcacattcaacaataaagaaaggtatctgtgcaacgccgatcacgtggccgccgccaacatcgccctgaccgtgaagggcatcggcgagcagagcagcgacgaggagaaccccgacggcagccgcatcaagctgcagctgaccagc

SEQ ID NO: 62 - DNA, 3162 bp, synthetic construct
  source 1..3162: mol_type = other DNA
atgagcagcgccatcaagagctacaagagcgtgctgcgccccaacgagcgcaagaaccagctgctgaagagcaccatccagtgcctggaggacggcagcgccttcttcttcaagatgctgcagggcctgttcggcggcatcacccccgagatcgtgcgcttcagcaccgagcaggagaagcagcagcaggacatcgccctgtggtgcgccgtgaactggttccgccccgtgagccaggacagcctgacccacaccatcgccagcgacaacctggtggagaagttcgaggagtactacggcggcaccgccagcgacgccatcaagcagtacttcagcgccagcatcggcgagagctactactggaacgactgccgccagcagtactacgacctgtgccgcgagctgggcgtggaggtgagcgacctgacccacgacctggagatcctgtgccgcgagaagtgcctggccgtggccaccgagagcaaccagtacaacagcatcatcagcgtgctgttcggcaccggcagaaaggaggaccgcagcgtgaagctgcgcatcaccaagaagatcctggaggccatcagcaacctgaaggagatccccaagaacgtggcccccatccaggagatcatcctgaacgtggccaaggccaccaaggagaccttccgccaggtgtacgccggcaacctgggcgcccccagcaccctggagagattcatcgccaaggacggccagaaggagttcgacctgaagaagctgcagaccgacctgaagaaggtgatccgcggcaagagcaaggagcgcgactggtgctgccaggaggagctgcgcagctacgtggagcagaacaccatccagtacgacctgtgggcctggggcgagatgttcaacaaggcccacaccgccctgaagatcaagagcacccgcaactacaacttcgccaagcagcgcctggagcagttcaagagaatccagagcctgaacaacctgctggtggtgaagaagctgaacgacttcttcgacagcgagttcttcagcggcgaggagacctacaccatctgcgtgcaccacctgggcggcaagagactgagcaagctgtacaaggcctgggaggacgaccccgccgaccccgagaacgccatcgtggtgctgtgcgacgacctgaagaacaacttcaagaaggagcccatccgcaacatcctgcgctacatcttcaccatccgccaggagtgcagcgcccaggacatcctggccgccgccaagtacaaccagcagctggaccgctacaagagccagaaggccaaccccagcgtgctgggcaaccagggcttcacctggagaaacgccgtgatcctgcccgagaaggcccagcgcaacgaccgccccaacagcctggacctgcgcatctggctgtacctgaagctgcgccaccccgacggccgctggaagaagcaccacatccccttctacgacacccgcttcttccaggagatctacgccgccggcaacagccccgtggacacctgccagttccgcaccccccgcttcggctaccacctgcccaagctgaccgaccagaccgccatccgcgtgaacaagaagcacgtgaaggccgccaagaccgaggcccgcatccgcctggccatccagcagggcaccctgcccgtgagcaacctgaagatcaccagaatcagcgccaccatcaacagcaagggccaggtgcgcatccccgtgaagttcgacgtgggccgccagaagggcaccctgcagatcggcgaccgcttctgcggctacgaccagaaccagaccgccagccacgcctacagcctgtgggaggtggtgaaggagggccagtaccacaaggagctgggctgcttcgtgcgcttcatcagcagcggcgacatcgtgagcatcaccgagaaccgcggcaaccagttcgaccagctgagctacgagggcctggcctacccccagtacgccgactggcgcaagaaggccagcaagttcgtgagcctgtggcagatcaccaagaagaacaagaagaaggagatcgtgaccgtggaggccaaggagaagttcgacgccatctgcaagtaccagccccgcctgtacaagttcaacaaggagtacgcctacctgctgcgcgacatcgtgcgcggcaagagcctggtggagctgcagcagatccgccaggagatcttccgcttcatcgagcaggactgcggcgtgacccgcctgggcagcctgagcctgagcaccctggagaccgtgaaggccgtgaagggcatcatctacagctacttcagcaccgccctgaacgccagcaagaacaaccccatcagcgacgagcagcgcaaggagttcgaccccgagctgttcgccctgctggagaagctggagctgatccgcacccgcaagaagaagcagaaggtggagcgcatcgccaacagcctgatccagacctgcctggagaacaacatcaagttcatccgcggcgagggcgacctgagcaccaccaacaacgccaccaagaagaaggccaacagccgcagcatggactggctggcccgcggcgtgttcaacaagatccgccagctggcccccatgcacaacatcaccctgttcggctgcggcagcctgtacaccagccaccaggaccccctggtgcaccgcaaccccgacaagtcttttagagctagatggagactcgtgaaggtcaaggacataggtgagaaggagctgctcaccctctccagaaacctgagagggaaagggaagggaataaagaagtactatcatcagggagtgctcgacttcttcaaggagtacgagctcgaagagctggccggaccactggccaagattaagcctggtgacccaaatgctataccacccgaggtcctgcggaataaactcaaagagaagctgggaaatgaagatgcaccagtgctgattcccgtcgccggaggcggcatctatctgagcactcacaatgtcgcaacaggcgccaagaagatcaccttcaataacaaagagcggtacgtctgcaacgccgatcacgtggccgccgccaacatcgccctgaccgtgaagggcatcggcgagcagagcagcgacgaggagaaccccgacggcagccgcatcaagctgcagctgaccagc

SEQ ID NO: 63 - DNA, 3162 bp, synthetic construct
  source 1..3162: mol_type = other DNA
atgagcagcgccatcaagagctacaagagcgtgctgcgccccaacgagcgcaagaaccagctgctgaagagcaccatccagtgcctggaggacggcagcgccttcttcttcaagatgctgcagggcctgttcggcggcatcacccccgagatcgtgcgcttcagcaccgagcaggagaagcagcagcaggacatcgccctgtggtgcgccgtgaactggttccgccccgtgagccaggacagcctgacccacaccatcgccagcgacaacctggtggagaagttcgaggagtactacggcggcaccgccagcgacgccatcaagcagtacttcagcgccagcatcggcgagagctactactggaacgactgccgccagcagtactacgacctgtgccgcgagctgggcgtggaggtgagcgacctgacccacgacctggagatcctgtgccgcgagaagtgcctggccgtggccaccgagagcaaccagtacaacagcatcatcagcgtgctgttcggcaccggcagaaaggaggaccgcagcgtgaagctgcgcatcaccaagaagatcctggaggccatcagcaacctgaaggagatccccaagaacgtggcccccatccaggagatcatcctgaacgtggccaaggccaccaaggagaccttccgccaggtgtacgccggcaacctgggcgcccccagcaccctggagagattcatcgccaaggacggccagaaggagttcgacctgaagaagctgcagaccgacctgaagaaggtgatccgcggcaagagcaaggagcgcgactggtgctgccaggaggagctgcgcagctacgtggagcagaacaccatccagtacgacctgtgggcctggggcgagatgttcaacaaggcccacaccgccctgaagatcaagagcacccgcaactacaacttcgccaagcagcgcctggagcagttcaagagaatccagagcctgaacaacctgctggtggtgaagaagctgaacgacttcttcgacagcgagttcttcagcggcgaggagacctacaccatctgcgtgcaccacctgggcggcaagagactgagcaagctgtacaaggcctgggaggacgaccccgccgaccccgagaacgccatcgtggtgctgtgcgacgacctgaagaacaacttcaagaaggagcccatccgcaacatcctgcgctacatcttcaccatccgccaggagtgcagcgcccaggacatcctggccgccgccaagtacaaccagcagctggaccgctacaagagccagaaggccaaccccagcgtgctgggcaaccagggcttcacctggagaaacgccgtgatcctgcccgagaaggcccagcgcaacgaccgccccaacagcctggacctgcgcatctggctgtacctgaagctgcgccaccccgacggccgctggaagaagcaccacatccccttctacgacacccgcttcttccaggagatctacgccgccggcaacagccccgtggacacctgccagttccgcaccccccgcttcggctaccacctgcccaagctgaccgaccagaccgccatccgcgtgaacaagaagcacgtgaaggccgccaagaccgaggcccgcatccgcctggccatccagcagggcaccctgcccgtgagcaacctgaagatcaccagaatcagcgccaccatcaacagcaagggccaggtgcgcatccccgtgaagttcgacgtgggccgccagaagggcaccctgcagatcggcgaccgcttctgcggctacgaccagaaccagaccgccagccacgcctacagcctgtgggaggtggtgaaggagggccagtaccacaaggagctgggctgcttcgtgcgcttcatcagcagcggcgacatcgtgagcatcaccgagaaccgcggcaaccagttcgaccagctgagctacgagggcctggcctacccccagtacgccgactggcgcaagaaggccagcaagttcgtgagcctgtggcagatcaccaagaagaacaagaagaaggagatcgtgaccgtggaggccaaggagaagttcgacgccatctgcaagtaccagccccgcctgtacaagttcaacaaggagtacgcctacctgctgcgcgacatcgtgcgcggcaagagcctggtggagctgcagcagatccgccaggagatcttccgcttcatcgagcaggactgcggcgtgacccgcctgggcagcctgagcctgagcaccctggagaccgtgaaggccgtgaagggcatcatctacagctacttcagcaccgccctgaacgccagcaagaacaaccccatcagcgacgagcagcgcaaggagttcgaccccgagctgttcgccctgctggagaagctggagctgatccgcacccgcaagaagaagcagaaggtggagcgcatcgccaacagcctgatccagacctgcctggagaacaacatcaagttcatccgcggcgagggcgacctgagcaccaccaacaacgccaccaagaagaaggccaacagccgcagcatggactggctggcccgcggcgtgttcaacaagatccgccagctggcccccatgcacaacatcaccctgttcggctgcggcagcctgtacaccagccaccaggaccccctggtgcaccgcaaccccgacaagaagtacaatgctcggtgggatctggttaaagtgaaggatattggtgagggccatctcctgattctgtcaagaaacctgcgcggcaaaggctctggcattaggaaatactaccatcagggcgtcctggagttctttaaagagtatgatctggaagatctggccgaacctctcgctaaaattagacccggtgatccaaacgccatccctcctgaagtgctcagagaacgcctcaaggagaagctcggcaacgaggacgctcctgttctcatccctaagcctggaggaggcgtgtacctcagcactcataacgtcgccaccggcgccaagaaaatcacattcaacaacaaggagagatacctgtgcaacgccgatcacgtggccgccgccaacatcgccctgaccgtgaagggcatcggcgagcagagcagcgacgaggagaaccccgacggcagccgcatcaagctgcagctgaccagc

SEQ ID NO: 64 - DNA, 3162 bp, synthetic construct
  source 1..3162: mol_type = other DNA
atgagcagcgccatcaagagctacaagagcgtgctgcgccccaacgagcgcaagaaccagctgctgaagagcaccatccagtgcctggaggacggcagcgccttcttcttcaagatgctgcagggcctgttcggcggcatcacccccgagatcgtgcgcttcagcaccgagcaggagaagcagcagcaggacatcgccctgtggtgcgccgtgaactggttccgccccgtgagccaggacagcctgacccacaccatcgccagcgacaacctggtggagaagttcgaggagtactacggcggcaccgccagcgacgccatcaagcagtacttcagcgccagcatcggcgagagctactactggaacgactgccgccagcagtactacgacctgtgccgcgagctgggcgtggaggtgagcgacctgacccacgacctggagatcctgtgccgcgagaagtgcctggccgtggccaccgagagcaaccagtacaacagcatcatcagcgtgctgttcggcaccggcagaaaggaggaccgcagcgtgaagctgcgcatcaccaagaagatcctggaggccatcagcaacctgaaggagatccccaagaacgtggcccccatccaggagatcatcctgaacgtggccaaggccaccaaggagaccttccgccaggtgtacgccggcaacctgggcgcccccagcaccctggagagattcatcgccaaggacggccagaaggagttcgacctgaagaagctgcagaccgacctgaagaaggtgatccgcggcaagagcaaggagcgcgactggtgctgccaggaggagctgcgcagctacgtggagcagaacaccatccagtacgacctgtgggcctggggcgagatgttcaacaaggcccacaccgccctgaagatcaagagcacccgcaactacaacttcgccaagcagcgcctggagcagttcaagagaatccagagcctgaacaacctgctggtggtgaagaagctgaacgacttcttcgacagcgagttcttcagcggcgaggagacctacaccatctgcgtgcaccacctgggcggcaagagactgagcaagctgtacaaggcctgggaggacgaccccgccgaccccgagaacgccatcgtggtgctgtgcgacgacctgaagaacaacttcaagaaggagcccatccgcaacatcctgcgctacatcttcaccatccgccaggagtgcagcgcccaggacatcctggccgccgccaagtacaaccagcagctggaccgctacaagagccagaaggccaaccccagcgtgctgggcaaccagggcttcacctggagaaacgccgtgatcctgcccgagaaggcccagcgcaacgaccgccccaacagcctggacctgcgcatctggctgtacctgaagctgcgccaccccgacggccgctggaagaagcaccacatccccttctacgacacccgcttcttccaggagatctacgccgccggcaacagccccgtggacacctgccagttccgcaccccccgcttcggctaccacctgcccaagctgaccgaccagaccgccatccgcgtgaacaagaagcacgtgaaggccgccaagaccgaggcccgcatccgcctggccatccagcagggcaccctgcccgtgagcaacctgaagatcaccagaatcagcgccaccatcaacagcaagggccaggtgcgcatccccgtgaagttcgacgtgggccgccagaagggcaccctgcagatcggcgaccgcttctgcggctacgaccagaaccagaccgccagccacgcctacagcctgtgggaggtggtgaaggagggccagtaccacaaggagctgggctgcttcgtgcgcttcatcagcagcggcgacatcgtgagcatcaccgagaaccgcggcaaccagttcgaccagctgagctacgagggcctggcctacccccagtacgccgactggcgcaagaaggccagcaagttcgtgagcctgtggcagatcaccaagaagaacaagaagaaggagatcgtgaccgtggaggccaaggagaagttcgacgccatctgcaagtaccagccccgcctgtacaagttcaacaaggagtacgcctacctgctgcgcgacatcgtgcgcggcaagagcctggtggagctgcagcagatccgccaggagatcttccgcttcatcgagcaggactgcggcgtgacccgcctgggcagcctgagcctgagcaccctggagaccgtgaaggccgtgaagggcatcatctacagctacttcagcaccgccctgaacgccagcaagaacaaccccatcagcgacgagcagcgcaaggagttcgaccccgagctgttcgccctgctggagaagctggagctgatccgcacccgcaagaagaagcagaaggtggagcgcatcgccaacagcctgatccagacctgcctggagaacaacatcaagttcatccgcggcgagggcgacctgagcaccaccaacaacgccaccaagaagaaggccaacagccgcagcatggactggctggcccgcggcgtgttcaacaagatccgccagctggcccccatgcacaacatcaccctgttcggctgcggcagcctgtacaccagccaccaggaccccctggtgcaccgcaaccccgacaagtcttatagagctaggtggagactggttagggttagagattttggcgagagacacctgctgaccctgtccagaaacctcaccgggaagggtaagggcaccaggaagtattatcatcagggcgtgctcgatttcttcagggaatacgatctggaggatctggctgggccactggctaaaataagaccaggcgaccctgatgccatacctcctgaagttctgcgggagcggctgcgggaaaagctcgggaacgacgaagctccagtgctcattcctgtgagaggaggtcctgtgtacctcagcacacatgatgttgcaaccggcgccaaaagaattacattcaatggcaaggagcgctacctgtgcaacgccgatcacgtggccgccgccaacatcgccctgaccgtgaagggcatcggcgagcagagcagcgacgaggagaaccccgacggcagccgcatcaagctgcagctgaccagc

SEQ ID NO: 65 - protein, 1044 aa, synthetic construct
MSSAIKSYKSVLRPNERKNQLLKSTIQCLEDGSAFFFKMLQGLFGGITPEIVRFSTEQEKQQQDIALWCAVNWFRPVSQDSLTHTIASDNLVEKFEEYYGGTASDAIKQYFSASIGESYYWNDCRQQYYDLCRELGVEVSDLTHDLEILCREKCLAVATESNQYNSIISVLFGTGRKEDRSVKLRITKKILEAISNLKEIPKNVAPIQEIILNVAKATKETFRQVYAGNLGAPSTLERFIAKDGQKEFDLKKLQTDLKKVIRGKSKERDWCCQEELRSYVEQNTIQYDLWAWGEMFNKAHTALKIKSTRNYNFAKQRLEQFKRIQSLNNLLVVKKLNDFFDSEFFSGEETYTICVHHLGGKRLSKLYKAWEDDPADPENAIVVLCDDLKNNFKKEPIRNILRYIFTIRQECSAQDILAAAKYNQQLDRYKSQKANPSVLGNQGFTWRNAVILPEKAQRNDRPNSLDLRIWLYLKLRHPDGRWKKHHIPFYDTRFFQEIYAAGNSPVDTCQFRTPRFGYHLPKLTDQTAIRVNKKHVKAAKTEARIRLAIQQGTLPVSNLKITRISATINSKGQVRIPVKFDVGRQKGTLQIGDRFCGYDQNQTASHAYSLWEVVKEGQYHKELGCFVRFISSGDIVSITENRGNQFDQLSYEGLAYPQYADWRKKASKFVSLWQITKKNKKKEIVTVEAKEKFDAICKYQPRLYKFNKEYAYLLRDIVRGKSLVELQQIRQEIFRFIEQDCGVTRLGSLSLSTLETVKAVKGIIYSYFSTALNASKNNPISDEQRKEFDPELFALLEKLELIRTRKKKQKVERIANSLIQTCLENNIKFIRGEGDLSTTNNATKKKANSRSMDWLARGVFNKIRQLAPMHNITLFGCGSLYTSHQDPLVHRNPDKAMRARFEEVNVENIAEWHVRNFSNYLRADSGTGLYYKQATMDFLKHYGLEEHAEGLENKKIKFYDFRKILEDKNLTSVIIPKRGGRIYMATNPVTSDSTPITYAGKTYNRCNAAHVAAANIALTVKGIGEQSSDEENPDGSRIKLQLTS

SEQ ID NO: 66 - protein, 1044 aa, synthetic construct
MSSAIKSYKSVLRPNERKNQLLKSTIQCLEDGSAFFFKMLQGLFGGITPEIVRFSTEQEKQQQDIALWCAVNWFRPVSQDSLTHTIASDNLVEKFEEYYGGTASDAIKQYFSASIGESYYWNDCRQQYYDLCRELGVEVSDLTHDLEILCREKCLAVATESNQYNSIISVLFGTGRKEDRSVKLRITKKILEAISNLKEIPKNVAPIQEIILNVAKATKETFRQVYAGNLGAPSTLERFIAKDGQKEFDLKKLQTDLKKVIRGKSKERDWCCQEELRSYVEQNTIQYDLWAWGEMFNKAHTALKIKSTRNYNFAKQRLEQFKRIQSLNNLLVVKKLNDFFDSEFFSGEETYTICVHHLGGKRLSKLYKAWEDDPADPENAIVVLCDDLKNNFKKEPIRNILRYIFTIRQECSAQDILAAAKYNQQLDRYKSQKANPSVLGNQGFTWRNAVILPEKAQRNDRPNSLDLRIWLYLKLRHPDGRWKKHHIPFYDTRFFQEIYAAGNSPVDTCQFRTPRFGYHLPKLTDQTAIRVNKKHVKAAKTEARIRLAIQQGTLPVSNLKITRISATINSKGQVRIPVKFDVGRQKGTLQIGDRFCGYDQNQTASHAYSLWEVVKEGQYHKELGCFVRFISSGDIVSITENRGNQFDQLSYEGLAYPQYADWRKKASKFVSLWQITKKNKKKEIVTVEAKEKFDAICKYQPRLYKFNKEYAYLLRDIVRGKSLVELQQIRQEIFRFIEQDCGVTRLGSLSLSTLETVKAVKGIIYSYFSTALNASKNNPISDEQRKEFDPELFALLEKLELIRTRKKKQKVERIANSLIQTCLENNIKFIRGEGDLSTTNNATKKKANSRSMDWLARGVFNKIRQLAPMHNITLFGCGSLYTSHQDPLVHRNPDKAMRARFEEVNVSNVSEWHMRNFSNYLRADSGTGLYYKQATLDFLKHYDLEEHADDLEKQNIKFYDFRKILEDKQLTSVIVPKRGGRIYMATNPVTSDSTPVTYAGKTYNRCNAAHVAAANIALTVKGIGEQSSDEENPDGSRIKLQLTS

SEQ ID NO: 67 - protein, 110 aa, synthetic construct
RARFEEVNVENIAEWHVRNFSNYLRADSGTGLYYKQATMDFLKHYGLEEHAEGLENKKIKFYDFRKILEDKNLTSVIIPKRGGRIYMATNPVTSDSTPITYAGKTYNRCN

SEQ ID NO: 68 - protein, 110 aa, synthetic construct
RARFEEVNVSNVSEWHMRNFSNYLRADSGTGLYYKQATLDFLKHYDLEEHADDLEKQNIKFYDFRKILEDKQLTSVIVPKRGGRIYMATNPVTSDSTPVTYAGKTYNRCN

SEQ ID NO: 69 - protein, 120 aa, synthetic construct
SFRARWDLVKVKDFGEKHLLTLSRNLTGKGPGTRKYYHQGVEDFLKEYELEDLKEELAKIKKGDPNALPPEVIRNKLKEKLGNENAPVLIPKRGGKYFLSTHNVATGAVKITFNNKERYL

SEQ ID NO: 70 - protein, 120 aa, synthetic construct
SFRARWRLVKVKDIGEKELLTLSRNLRGKGKGIKKYYHQGVLDFFKEYELEELAGPLAKIKPGDPNAIPPEVLRNKLKEKLGNEDAPVLIPVAGGGIYLSTHNVATGAKKITFNNKERYV

SEQ ID NO: 71 - protein, 120 aa, synthetic construct
KYNARWDLVKVKDIGEGHLLILSRNLRGKGSGIRKYYHQGVLEFFKEYDLEDLAEPLAKIRPGDPNAIPPEVLRERLKEKLGNEDAPVLIPKPGGGVYLSTHNVATGAKKITFNNKERYL

SEQ ID NO: 72 - protein, 120 aa, synthetic construct
SYRARWRLVRVRDFGERHLLTLSRNLTGKGKGTRKYYHQGVLDFFREYDLEDLAGPLAKIRPGDPDAIPPEVLRERLREKLGNDEAPVLIPVRGGPVYLSTHDVATGAKRITFNGKERYL

SEQ ID NO: 73 - RNA, 20 nt, synthetic construct
  source 1..20: mol_type = other RNA
aggccaaagaattcctggaa

SEQ ID NO: 74 - RNA, 20 nt, synthetic construct
  source 1..20: mol_type = other RNA
tcacaggctccaggaagggt

SEQ ID NO: 75 - RNA, 20 nt, synthetic construct
  source 1..20: mol_type = other RNA
ttcaacatatccaaacaaat

SEQ ID NO: 76 - DNA, 22 bp, synthetic construct
  source 1..22: mol_type = other DNA
tctgcttcggtgtcgaaatgag

SEQ ID NO: 77 - DNA, 22 bp, synthetic construct
  source 1..22: mol_type = other DNA
tgcagaagcgtttggcaatgtg

SEQ ID NO: 78 - DNA, 20 bp, synthetic construct
  source 1..20: mol_type = other DNA
gctgaaaagcgatacagggc

SEQ ID NO: 79 - DNA, 20 bp, synthetic construct
  source 1..20: mol_type = other DNA
atcaccaagagagccttccg

SEQ ID NO: 80 - DNA, 23 bp, synthetic construct
  source 1..23: mol_type = other DNA
tttataacagtggtggtgaggct

SEQ ID NO: 81 - DNA, 22 bp, synthetic construct
  source 1..22: mol_type = other DNA
ttctcaaaccctggaaagcact

SEQ ID NO: 82 - RNA, 20 nt, synthetic construct
  source 1..20: mol_type = other RNA
atttgtttggatatgttgaa

SEQ ID NO: 83 - protein, 32 aa, synthetic construct
SGGSSGGSSGSETPGTSESATPESSGGSSGGS

SEQ ID NO: 84 - RNA, 20 nt, synthetic construct
  source 1..20: mol_type = other RNA
ttgtataataggaaagggaa

SEQ ID NO: 85 - RNA, 20 nt, synthetic construct
  source 1..20: mol_type = other RNA
tctatcactgatagggagtg

SEQ ID NO: 86 - protein, 80 aa, synthetic construct
GGPSSGAPPPSGGSPAGSPTSTEEGTSESATPESGPGTSTEPSEGSAPGSPAGSPTSTEEGTSTEPSEGSAPGTSTEPSE

SEQ ID NO: 87 - protein, 10 aa, synthetic construct
SGGSGGSGGS

SEQ ID NO: 88 - protein, 1598 aa, synthetic construct
PKKKRKVMSSAIKSYKSVLRPNERKNQLLKSTIQCLEDGSAFFFKMLQGLFGGITPEIVRFSTEQEKQQQDIALWCAVNWFRPVSQDSLTHTIASDNLVEKFEEYYGGTASDAIKQYFSASIGESYYWNDCRQQYYDLCRELGVEVSDLTHDLEILCREKCLAVATESNQYNSIISVLFGTGRKEDRSVKLRITKKILEAISNLKEIPKNVAPIQEIILNVAKATKETFRQVYAGNLGAPSTLERFIAKDGQKEFDLKKLQTDLKKVIRGKSKERDWCCQEELRSYVEQNTIQYDLWAWGEMFNKAHTALKIKSTRNYNFAKQRLEQFKRIQSLNNLLVVKKLNDFFDSEFFSGEETYTICVHHLGGKRLSKLYKAWEDDPADPENAIVVLCDDLKNNFKKEPIRNILRYIFTIRQECSAQDILAAAKYNQQLDRYKSQKANPSVLGNQGFTWRNAVILPEKAQRNDRPNSLDLRIWLYLKLRHPDGRWKKHHIPFYDTRFFQEIYAAGNSPVDTCQFRTPRFGYHLPKLTDQTAIRVNKKHVKAAKTEARIRLAIQQGTLPVSNLKITRISATINSKGQVRIPVKFDVGRQKGTLQIGDRFCGYDQNQTASHAYSLWEVVKEGQYHKELGCFVRFISSGDIVSITENRGNQFDQLSYEGLAYPQYADWRKKASKFVSLWQITKKNKKKEIVTVEAKEKFDAICKYQPRLYKFNKEYAYLLRDIVRGKSLVELQQIRQEIFRFIEQDCGVTRLGSLSLSTLETVKAVKGIIYSYFSTALNASKNNPISDEQRKEFDPELFALLEKLELIRTRKKKQKVERIANSLIQTCLENNIKFIRGEGDLSTTNNATKKKANSRSMDWLARGVFNKIRQLAPMHNITLFGCGSLYTSHQDPLVHRNPDKAMRARFEEVNVENIAEWHVRNFSNYLRADSGTGLYYKQATMDFLKHYGLEEHAEGLENKKIKFYDFRKILEDKNLTSVIIPKRGGRIYMATNPVTSDSTPITYAGKTYNRCNAAHVAAANIALTVKGIGEQSSDEENPDGSRIKLQLTSKRPAATKKAGQAKKKKEASGSGRADALDDFDLDMLGSDALDDFDLDMLGSDALDDFDLDMLGSDALDDFDLDMLINSRSSGSPKKKRKVGSQYLPDTDDRHRIEEKRKRTYETFKSIMKKSPFSGPTDPRPPPRRIAVPSRSSASVPKPAPQPYPFTSSLSTINYDEFPTMVFPSGQISQASALAPAPPQVLPQAPAPAPAPAMVSALAQAPAPVPVLAPGPPQAVAPPAPKPTQAGEGTLSEALLQLQFDDEDLGALLGNSTDPAVFTDLASVDNSEFQQLLNQGIPVAPHTTEPMLMEYPEAITRLVTGAQRPPDPAPAPLGAPGLPNGLLSGDEDFSSIADMDFSALLGSGSGSRDSREGMFLPKPEAGSAISDVFEGREVCQPKRIRPFHPPGSPWANRPLPASLAPTPTGPVHEPVGSLTPAPVPQPLDPAPAVTPEASHLLEDPDEETSQAVKALREMADTVIPQKEEAAICGQMDLSHPPPRGHLDELTTTLESMTEDLNLDSPLTPELNEILDTFLNDECLLHAMHISTGLSIFDTSLF

SEQ ID NO: 89 - protein, 1598 aa, synthetic construct
PKKKRKVMSSAIKSYKSVLRPNERKNQLLKSTIQCLEDGSAFFFKMLQGLFGGITPEIVRFSTEQEKQQQDIALWCAVNWFRPVSQDSLTHTIASDNLVEKFEEYYGGTASDAIKQYFSASIGESYYWNDCRQQYYDLCRELGVEVSDLTHDLEILCREKCLAVATESNQYNSIISVLFGTGRKEDRSVKLRITKKILEAISNLKEIPKNVAPIQEIILNVAKATKETFRQVYAGNLGAPSTLERFIAKDGQKEFDLKKLQTDLKKVIRGKSKERDWCCQEELRSYVEQNTIQYDLWAWGEMFNKAHTALKIKSTRNYNFAKQRLEQFKRIQSLNNLLVVKKLNDFFDSEFFSGEETYTICVHHLGGKRLSKLYKAWEDDPADPENAIVVLCDDLKNNFKKEPIRNILRYIFTIRQECSAQDILAAAKYNQQLDRYKSQKANPSVLGNQGFTWRNAVILPEKAQRNDRPNSLDLRIWLYLKLRHPDGRWKKHHIPFYDTRFFQEIYAAGNSPVDTCQFRTPRFGYHLPKLTDQTAIRVNKKHVKAAKTEARIRLAIQQGTLPVSNLKITRISATINSKGQVRIPVKFDVGRQKGTLQIGDRFCGYDQNQTASHAYSLWEVVKEGQYHKELGCFVRFISSGDIVSITENRGNQFDQLSYEGLAYPQYADWRKKASKFVSLWQITKKNKKKEIVTVEAKEKFDAICKYQPRLYKFNKEYAYLLRDIVRGKSLVELQQIRQEIFRFIEQDCGVTRLGSLSLSTLETVKAVKGIIYSYFSTALNASKNNPISDEQRKEFDPELFALLEKLELIRTRKKKQKVERIANSLIQTCLENNIKFIRGEGDLSTTNNATKKKANSRSMDWLARGVFNKIRQLAPMHNITLFGCGSLYTSHQDPLVHRNPDKAMRARFEEVNVSNVSEWHMRNFSNYLRADSGTGLYYKQATLDFLKHYDLEEHADDLEKQNIKFYDFRKILEDKQLTSVIVPKRGGRIYMATNPVTSDSTPVTYAGKTYNRCNAAHVAAANIALTVKGIGEQSSDEENPDGSRIKLQLTSKRPAATKKAGQAKKKKEASGSGRADALDDFDLDMLGSDALDDFDLDMLGSDALDDFDLDMLGSDALDDFDLDMLINSRSSGSPKKKRKVGSQYLPDTDDRHRIEEKRKRTYETFKSIMKKSPFSGPTDPRPPPRRIAVPSRSSASVPKPAPQPYPFTSSLSTINYDEFPTMVFPSGQISQASALAPAPPQVLPQAPAPAPAPAMVSALAQAPAPVPVLAPGPPQAVAPPAPKPTQAGEGTLSEALLQLQFDDEDLGALLGNSTDPAVFTDLASVDNSEFQQLLNQGIPVAPHTTEPMLMEYPEAITRLVTGAQRPPDPAPAPLGAPGLPNGLLSGDEDFSSIADMDFSALLGSGSGSRDSREGMFLPKPEAGSAISDVFEGREVCQPKRIRPFHPPGSPWANRPLPASLAPTPTGPVHEPVGSLTPAPVPQPLDPAPAVTPEASHLLEDPDEETSQAVKALREMADTVIPQKEEAAICGQMDLSHPPPRGHLDELTTTLESMTEDLNLDSPLTPELNEILDTFLNDECLLHAMHISTGLSIFDTSLF

SEQ ID NO: 90 - protein, 1380 aa, synthetic construct
PKKKRKVMSSAIKSYKSVLRPNERKNQLLKSTIQCLEDGSAFFFKMLQGLFGGITPEIVRFSTEQEKQQQDIALWCAVNWFRPVSQDSLTHTIASDNLVEKFEEYYGGTASDAIKQYFSASIGESYYWNDCRQQYYDLCRELGVEVSDLTHDLEILCREKCLAVATESNQYNSIISVLFGTGRKEDRSVKLRITKKILEAISNLKEIPKNVAPIQEIILNVAKATKETFRQVYAGNLGAPSTLERFIAKDGQKEFDLKKLQTDLKKVIRGKSKERDWCCQEELRSYVEQNTIQYDLWAWGEMFNKAHTALKIKSTRNYNFAKQRLEQFKRIQSLNNLLVVKKLNDFFDSEFFSGEETYTICVHHLGGKRLSKLYKAWEDDPADPENAIVVLCDDLKNNFKKEPIRNILRYIFTIRQECSAQDILAAAKYNQQLDRYKSQKANPSVLGNQGFTWRNAVILPEKAQRNDRPNSLDLRIWLYLKLRHPDGRWKKHHIPFYDTRFFQEIYAAGNSPVDTCQFRTPRFGYHLPKLTDQTAIRVNKKHVKAAKTEARIRLAIQQGTLPVSNLKITRISATINSKGQVRIPVKFDVGRQKGTLQIGDRFCGYDQNQTASHAYSLWEVVKEGQYHKELGCFVRFISSGDIVSITENRGNQFDQLSYEGLAYPQYADWRKKASKFVSLWQITKKNKKKEIVTVEAKEKFDAICKYQPRLYKFNKEYAYLLRDIVRGKSLVELQQIRQEIFRFIEQDCGVTRLGSLSLSTLETVKAVKGIIYSYFSTALNASKNNPISDEQRKEFDPELFALLEKLELIRTRKKKQKVERIANSLIQTCLENNIKFIRGEGDLSTTNNATKKKANSRSMDWLARGVFNKIRQLAPMHNITLFGCGSLYTSHQDPLVHRNPDKAMRARFEEVNVENIAEWHVRNFSNYLRADSGTGLYYKQATMDFLKHYGLEEHAEGLENKKIKFYDFRKILEDKNLTSVIIPKRGGRIYMATNPVTSDSTPITYAGKTYNRCNAAHVAAANIALTVKGIGEQSSDEENPDGSRIKLQLTSKRPAATKKAGQAKKKKDALDDFDLDMLGSDALDDFDLDMLGSDALDDFDLDMLGSDALDDFDLDMLINSRSSGSPKKKRKVGSGGGSGGSGSVLPQAPAPAPAPAMVSALAQAPAPVPVLAPGPPQAVAPPAPKPTQAGEGTLSEALLQLQFDDEDLGALLGNSTDPAVFTDLASVDNSEFQQLLNQGIPVAPHTTEPMLMEYPEAITRLVTGAQRPPDPAPAPLGAPGLPNGLLSGDEDFSSIADMDFSALLSGGGSGGSGSDLSHPPPRGHLDELTTTLESMTEDLNLDSPLTPELNEILDTFLNDECLLHAMHISTGLSIFDTSLF

SEQ ID NO: 91 - protein, 1380 aa, synthetic construct
PKKKRKVMSSAIKSYKSVLRPNERKNQLLKSTIQCLEDGSAFFFKMLQGLFGGITPEIVRFSTEQEKQQQDIALWCAVNWFRPVSQDSLTHTIASDNLVEKFEEYYGGTASDAIKQYFSASIGESYYWNDCRQQYYDLCRELGVEVSDLTHDLEILCREKCLAVATESNQYNSIISVLFGTGRKEDRSVKLRITKKILEAISNLKEIPKNVAPIQEIILNVAKATKETFRQVYAGNLGAPSTLERFIAKDGQKEFDLKKLQTDLKKVIRGKSKERDWCCQEELRSYVEQNTIQYDLWAWGEMFNKAHTALKIKSTRNYNFAKQRLEQFKRIQSLNNLLVVKKLNDFFDSEFFSGEETYTICVHHLGGKRLSKLYKAWEDDPADPENAIVVLCDDLKNNFKKEPIRNILRYIFTIRQECSAQDILAAAKYNQQLDRYKSQKANPSVLGNQGFTWRNAVILPEKAQRNDRPNSLDLRIWLYLKLRHPDGRWKKHHIPFYDTRFFQEIYAAGNSPVDTCQFRTPRFGYHLPKLTDQTAIRVNKKHVKAAKTEARIRLAIQQGTLPVSNLKITRISATINSKGQVRIPVKFDVGRQKGTLQIGDRFCGYDQNQTASHAYSLWEVVKEGQYHKELGCFVRFISSGDIVSITENRGNQFDQLSYEGLAYPQYADWRKKASKFVSLWQITKKNKKKEIVTVEAKEKFDAICKYQPRLYKFNKEYAYLLRDIVRGKSLVELQQIRQEIFRFIEQDCGVTRLGSLSLSTLETVKAVKGIIYSYFSTALNASKNNPISDEQRKEFDPELFALLEKLELIRTRKKKQKVERIANSLIQTCLENNIKFIRGEGDLSTTNNATKKKANSRSMDWLARGVFNKIRQLAPMHNITLFGCGSLYTSHQDPLVHRNPDKAMRARFEEVNVSNVSEWHMRNFSNYLRADSGTGLYYKQATLDFLKHYDLEEHADDLEKQNIKFYDFRKILEDKQLTSVIVPKRGGRIYMATNPVTSDSTPVTYAGKTYNRCNAAHVAAANIALTVKGIGEQSSDEENPDGSRIKLQLTSKRPAATKKAGQAKKKKDALDDFDLDMLGSDALDDFDLDMLGSDALDDFDLDMLGSDALDDFDLDMLINSRSSGSPKKKRKVGSGGGSGGSGSVLPQAPAPAPAPAMVSALAQAPAPVPVLAPGPPQAVAPPAPKPTQAGEGTLSEALLQLQFDDEDLGALLGNSTDPAVFTDLASVDNSEFQQLLNQGIPVAPHTTEPMLMEYPEAITRLVTGAQRPPDPAPAPLGAPGLPNGLLSGDEDFSSIADMDFSALLSGGGSGGSGSDLSHPPPRGHLDELTTTLESMTEDLNLDSPLTPELNEILDTFLNDECLLHAMHISTGLSIFDTSLF

SEQ ID NO: 92 - protein, 1765 aa, synthetic construct
MNHDQEFDPPKVYPPVPAEKRKPIRVLSLFDGIATGLLVLKDLGIQVDRYIASEVCEDSITVGMVRHQGKIMYVGDVRSVTQKHIQEWGPFDLVIGGSPCNDLSIVNPARKGLYEGTGRLFFEFYRLLHDARPKEGDDRPFFWLFENVVAMGVSDKRDISRFLESNPVMIDAKEVSAAHRARYFWGNLPGMNRPLASTVNDKLELQECLEHGRIAKFSKVRTITTRSNSIKQGKDQHFPVFMNEKEDILWCTEMERVFGFPVHYTDVSNMSRLARQRLLGRSWSVPVIRHLFAPLKEYFACVSSGNSNANSRGPSFSSGLVPLSLRGSHMGPMEIYKTVSAWKRQPVRVLSLFRNIDKVLKSLGFLESGSGSGGGTLKYVEDVTNVVRRDVEKWGPFDLVYGSTQPLGSSCDRCPGWYMFQFHRILQYALPRQESQRPFFWIFMDNLLLTEDDQETTTRFLQTEAVTLQDVRGRDYQNAMRVWSNIPGLKSKHAPLTPKEEEYLQAQVRSRSKLDAPKVDLLVKNCLLPLREYFKYFSQNSLPLGGPSSGAPPPSGGSPAGSPTSTEEGTSESATPESGPGTSTEPSEGSAPGSPAGSPTSTEEGTSTEPSEGSAPGTSTEPSEMSSAIKSYKSVLRPNERKNQLLKSTIQCLEDGSAFFFKMLQGLFGGITPEIVRFSTEQEKQQQDIALWCAVNWFRPVSQDSLTHTIASDNLVEKFEEYYGGTASDAIKQYFSASIGESYYWNDCRQQYYDLCRELGVEVSDLTHDLEILCREKCLAVATESNQYNSIISVLFGTGRKEDRSVKLRITKKILEAISNLKEIPKNVAPIQEIILNVAKATKETFRQVYAGNLGAPSTLERFIAKDGQKEFDLKKLQTDLKKVIRGKSKERDWCCQEELRSYVEQNTIQYDLWAWGEMFNKAHTALKIKSTRNYNFAKQRLEQFKRIQSLNNLLVVKKLNDFFDSEFFSGEETYTICVHHLGGKRLSKLYKAWEDDPADPENAIVVLCDDLKNNFKKEPIRNILRYIFTIRQECSAQDILAAAKYNQQLDRYKSQKANPSVLGNQGFTWRNAVILPEKAQRNDRPNSLDLRIWLYLKLRHPDGRWKKHHIPFYDTRFFQEIYAAGNSPVDTCQFRTPRFGYHLPKLTDQTAIRVNKKHVKAAKTEARIRLAIQQGTLPVSNLKITRISATINSKGQVRIPVKFDVGRQKGTLQIGDRFCGYDQNQTASHAYSLWEVVKEGQYHKELGCFVRFISSGDIVSITENRGNQFDQLSYEGLAYPQYADWRKKASKFVSLWQITKKNKKKEIVTVEAKEKFDAICKYQPRLYKFNKEYAYLLRDIVRGKSLVELQQIRQEIFRFIEQDCGVTRLGSLSLSTLETVKAVKGIIYSYFSTALNASKNNPISDEQRKEFDPELFALLEKLELIRTRKKKQKVERIANSLIQTCLENNIKFIRGEGDLSTTNNATKKKANSRSMDWLARGVFNKIRQLAPMHNITLFGCGSLYTSHQDPLVHRNPDKAMRARFEEVNVENIAEWHVRNFSNYLRADSGTGLYYKQATMDFLKHYGLEEHAEGLENKKIKFYDFRKILEDKNLTSVIIPKRGGRIYMATNPVTSDSTPITYAGKTYNRCNAAHVAAANIALTVKGIGEQSSDEENPDGSRIKLQLTSPKKKRKVDGIGSGSNGSSGSGGGGGMDAKSLTAWSRTLVTFKDVFVDFTREEWKLLDTAQQIVYRNVMLENYKNLVSLGYQLTKPDVILRLEKGEEP

SEQ ID NO: 93 - protein, 1765 aa, synthetic construct
MNHDQEFDPPKVYPPVPAEKRKPIRVLSLFDGIATGLLVLKDLGIQVDRYIASEVCEDSITVGMVRHQGKIMYVGDVRSVTQKHIQEWGPFDLVIGGSPCNDLSIVNPARKGLYEGTGRLFFEFYRLLHDARPKEGDDRPFFWLFENVVAMGVSDKRDISRFLESNPVMIDAKEVSAAHRARYFWGNLPGMNRPLASTVNDKLELQECLEHGRIAKFSKVRTITTRSNSIKQGKDQHFPVFMNEKEDILWCTEMERVFGFPVHYTDVSNMSRLARQRLLGRSWSVPVIRHLFAPLKEYFACVSSGNSNANSRGPSFSSGLVPLSLRGSHMGPMEIYKTVSAWKRQPVRVLSLFRNIDKVLKSLGFLESGSGSGGGTLKYVEDVTNVVRRDVEKWGPFDLVYGSTQPLGSSCDRCPGWYMFQFHRILQYALPRQESQRPFFWIFMDNLLLTEDDQETTTRFLQTEAVTLQDVRGRDYQNAMRVWSNIPGLKSKHAPLTPKEEEYLQAQVRSRSKLDAPKVDLLVKNCLLPLREYFKYFSQNSLPLGGPSSGAPPPSGGSPAGSPTSTEEGTSESATPESGPGTSTEPSEGSAPGSPAGSPTSTEEGTSTEPSEGSAPGTSTEPSEMSSAIKSYKSVLRPNERKNQLLKSTIQCLEDGSAFFFKMLQGLFGGITPEIVRFSTEQEKQQQDIALWCAVNWFRPVSQDSLTHTIASDNLVEKFEEYYGGTASDAIKQYFSASIGESYYWNDCRQQYYDLCRELGVEVSDLTHDLEILCREKCLAVATESNQYNSIISVLFGTGRKEDRSVKLRITKKILEAISNLKEIPKNVAPIQEIILNVAKATKETFRQVYAGNLGAPSTLERFIAKDGQKEFDLKKLQTDLKKVIRGKSKERDWCCQEELRSYVEQNTIQYDLWAWGEMFNKAHTALKIKSTRNYNFAKQRLEQFKRIQSLNNLLVVKKLNDFFDSEFFSGEETYTICVHHLGGKRLSKLYKAWEDDPADPENAIVVLCDDLKNNFKKEPIRNILRYIFTIRQECSAQDILAAAKYNQQLDRYKSQKANPSVLGNQGFTWRNAVILPEKAQRNDRPNSLDLRIWLYLKLRHPDGRWKKHHIPFYDTRFFQEIYAAGNSPVDTCQFRTPRFGYHLPKLTDQTAIRVNKKHVKAAKTEARIRLAIQQGTLPVSNLKITRISATINSKGQVRIPVKFDVGRQKGTLQIGDRFCGYDQNQTASHAYSLWEVVKEGQYHKELGCFVRFISSGDIVSITENRGNQFDQLSYEGLAYPQYADWRKKASKFVSLWQITKKNKKKEIVTVEAKEKFDAICKYQPRLYKFNKEYAYLLRDIVRGKSLVELQQIRQEIFRFIEQDCGVTRLGSLSLSTLETVKAVKGIIYSYFSTALNASKNNPISDEQRKEFDPELFALLEKLELIRTRKKKQKVERIANSLIQTCLENNIKFIRGEGDLSTTNNATKKKANSRSMDWLARGVFNKIRQLAPMHNITLFGCGSLYTSHQDPLVHRNPDKAMRARFEEVNVSNVSEWHMRNFSNYLRADSGTGLYYKQATLDFLKHYDLEEHADDLEKQNIKFYDFRKILEDKQLTSVIVPKRGGRIYMATNPVTSDSTPVTYAGKTYNRCNAAHVAAANIALTVKGIGEQSSDEENPDGSRIKLQLTSPKKKRKVDGIGSGSNGSSGSGGGGGMDAKSLTAWSRTLVTFKDVFVDFTREEWKLLDTAQQIVYRNVMLENYKNLVSLGYQLTKPDVILRLEKGEEP

SEQ ID NO: 94 - protein, 1249 aa, synthetic construct
PKKKRKVSEVEFSHEYWMRHALTLAKRARDEREVPVGAVLVLNNRVIGEGWNRAIGLHDPTAHAEIMALRQGGLVMQNYRLIDATLYVTFEPCVMCAGAMIHSRIGRVVFGVRNSKRGAAGSLMNVLNYPGMNHRVEITEGILADECAALLCDFYRMPRQVFNAQKKAQSSINSGGSSGGSSGSETPGTSESATPESSGGSSGGSMSSAIKSYKSVLRPNERKNQLLKSTIQCLEDGSAFFFKMLQGLFGGITPEIVRFSTEQEKQQQDIALWCAVNWFRPVSQDSLTHTIASDNLVEKFEEYYGGTASDAIKQYFSASIGESYYWNDCRQQYYDLCRELGVEVSDLTHDLEILCREKCLAVATESNQYNSIISVLFGTGRKEDRSVKLRITKKILEAISNLKEIPKNVAPIQEIILNVAKATKETFRQVYAGNLGAPSTLERFIAKDGQKEFDLKKLQTDLKKVIRGKSKERDWCCQEELRSYVEQNTIQYDLWAWGEMFNKAHTALKIKSTRNYNFAKQRLEQFKRIQSLNNLLVVKKLNDFFDSEFFSGEETYTICVHHLGGKRLSKLYKAWEDDPADPENAIVVLCDDLKNNFKKEPIRNILRYIFTIRQECSAQDILAAAKYNQQLDRYKSQKANPSVLGNQGFTWRNAVILPEKAQRNDRPNSLDLRIWLYLKLRHPDGRWKKHHIPFYDTRFFQEIYAAGNSPVDTCQFRTPRFGYHLPKLTDQTAIRVNKKHVKAAKTEARIRLAIQQGTLPVSNLKITRISATINSKGQVRIPVKFDVGRQKGTLQIGDRFCGYDQNQTASHAYSLWEVVKEGQYHKELGCFVRFISSGDIVSITENRGNQFDQLSYEGLAYPQYADWRKKASKFVSLWQITKKNKKKEIVTVEAKEKFDAICKYQPRLYKFNKEYAYLLRDIVRGKSLVELQQIRQEIFRFIEQDCGVTRLGSLSLSTLETVKAVKGIIYSYFSTALNASKNNPISDEQRKEFDPELFALLEKLELIRTRKKKQKVERIANSLIQTCLENNIKFIRGEGDLSTTNNATKKKANSRSMDWLARGVFNKIRQLAPMHNITLFGCGSLYTSHQDPLVHRNPDKAMRARFEEVNVENIAEWHVRNFSNYLRADSGTGLYYKQATMDFLKHYGLEEHAEGLENKKIKFYDFRKILEDKNLTSVIIPKRGGRIYMATNPVTSDSTPITYAGKTYNRCNAAHVAAANIALTVKGIGEQSSDEENPDGSRIKLQLTS

SEQ ID NO: 95 - protein, 1249 aa, synthetic construct
PKKKRKVSEVEFSHEYWMRHALTLAKRARDEREVPVGAVLVLNNRVIGEGWNRAIGLHDPTAHAEIMALRQGGLVMQNYRLIDATLYVTFEPCVMCAGAMIHSRIGRVVFGVRNSKRGAAGSLMNVLNYPGMNHRVEITEGILADECAALLCDFYRMPRQVFNAQKKAQSSINSGGSSGGSSGSETPGTSESATPESSGGSSGGSMSSAIKSYKSVLRPNERKNQLLKSTIQCLEDGSAFFFKMLQGLFGGITPEIVRFSTEQEKQQQDIALWCAVNWFRPVSQDSLTHTIASDNLVEKFEEYYGGTASDAIKQYFSASIGESYYWNDCRQQYYDLCRELGVEVSDLTHDLEILCREKCLAVATESNQYNSIISVLFGTGRKEDRSVKLRITKKILEAISNLKEIPKNVAPIQEIILNVAKATKETFRQVYAGNLGAPSTLERFIAKDGQKEFDLKKLQTDLKKVIRGKSKERDWCCQEELRSYVEQNTIQYDLWAWGEMFNKAHTALKIKSTRNYNFAKQRLEQFKRIQSLNNLLVVKKLNDFFDSEFFSGEETYTICVHHLGGKRLSKLYKAWEDDPADPENAIVVLCDDLKNNFKKEPIRNILRYIFTIRQECSAQDILAAAKYNQQLDRYKSQKANPSVLGNQGFTWRNAVILPEKAQRNDRPNSLDLRIWLYLKLRHPDGRWKKHHIPFYDTRFFQEIYAAGNSPVDTCQFRTPRFGYHLPKLTDQTAIRVNKKHVKAAKTEARIRLAIQQGTLPVSNLKITRISATINSKGQVRIPVKFDVGRQKGTLQIGDRFCGYDQNQTASHAYSLWEVVKEGQYHKELGCFVRFISSGDIVSITENRGNQFDQLSYEGLAYPQYADWRKKASKFVSLWQITKKNKKKEIVTVEAKEKFDAICKYQPRLYKFNKEYAYLLRDIVRGKSLVELQQIRQEIFRFIEQDCGVTRLGSLSLSTLETVKAVKGIIYSYFSTALNASKNNPISDEQRKEFDPELFALLEKLELIRTRKKKQKVERIANSLIQTCLENNIKFIRGEGDLSTTNNATKKKANSRSMDWLARGVFNKIRQLAPMHNITLFGCGSLYTSHQDPLVHRNPDKAMRARFEEVNVSNVSEWHMRNFSNYLRADSGTGLYYKQATLDFLKHYDLEEHADDLEKQNIKFYDFRKILEDKQLTSVIVPKRGGRIYMATNPVTSDSTPVTYAGKTYNRCNAAHVAAANIALTVKGIGEQSSDEENPDGSRIKLQLTS

SEQ ID NO: 96 - protein, 1497 aa, synthetic construct
PKKKRKVSSETGPVAVDPTLRRRIEPHEFEVFFDPRELRKETCLLYEINWGGRHSIWRHTSQNTNKHVEVNFIEKFTTERYFCPNTRCSITWFLSWSPCGECSRAITEFLSRYPHVTLFIYIARLYHHADPRNRQGLRDLISSGVTIQIMTEQESGYCWRNFVNYSPSNEAHWPRYPHLWVRLYVLELYCIILGLPPCLNILRRKQPQLTFFTIALQSCHYQRLPPHILWATGLKSGGSSGGSSGSETPGTSESATPESSGGSSGGSMSSAIKSYKSVLRPNERKNQLLKSTIQCLEDGSAFFFKMLQGLFGGITPEIVRFSTEQEKQQQDIALWCAVNWFRPVSQDSLTHTIASDNLVEKFEEYYGGTASDAIKQYFSASIGESYYWNDCRQQYYDLCRELGVEVSDLTHDLEILCREKCLAVATESNQYNSIISVLFGTGRKEDRSVKLRITKKILEAISNLKEIPKNVAPIQEIILNVAKATKETFRQVYAGNLGAPSTLERFIAKDGQKEFDLKKLQTDLKKVIRGKSKERDWCCQEELRSYVEQNTIQYDLWAWGEMFNKAHTALKIKSTRNYNFAKQRLEQFKRIQSLNNLLVVKKLNDFFDSEFFSGEETYTICVHHLGGKRLSKLYKAWEDDPADPENAIVVLCDDLKNNFKKEPIRNILRYIFTIRQECSAQDILAAAKYNQQLDRYKSQKANPSVLGNQGFTWRNAVILPEKAQRNDRPNSLDLRIWLYLKLRHPDGRWKKHHIPFYDTRFFQEIYAAGNSPVDTCQFRTPRFGYHLPKLTDQTAIRVNKKHVKAAKTEARIRLAIQQGTLPVSNLKITRISATINSKGQVRIPVKFDVGRQKGTLQIGDRFCGYDQNQTASHAYSLWEVVKEGQYHKELGCFVRFISSGDIVSITENRGNQFDQLSYEGLAYPQYADWRKKASKFVSLWQITKKNKKKEIVTVEAKEKFDAICKYQPRLYKFNKEYAYLLRDIVRGKSLVELQQIRQEIFRFIEQDCGVTRLGSLSLSTLETVKAVKGIIYSYFSTALNASKNNPISDEQRKEFDPELFALLEKLELIRTRKKKQKVERIANSLIQTCLENNIKFIRGEGDLSTTNNATKKKANSRSMDWLARGVFNKIRQLAPMHNITLFGCGSLYTSHQDPLVHRNPDKAMRARFEEVNVENIAEWHVRNFSNYLRADSGTGLYYKQATMDFLKHYGLEEHAEGLENKKIKFYDFRKILEDKNLTSVIIPKRGGRIYMATNPVTSDSTPITYAGKTYNRCNAAHVAAANIALTVKGIGEQSSDEENPDGSRIKLQLTSSGGSGGSGGSTNLSDIIEKETGKQLVIQESILMLPEEVEEVIGNKPESDILVHTAYDESTDENVMLLTSDAPEYKPWALVIQDSNGENKIKMLSGGSGGSGGSTNLSDIIEKETGKQLVIQESILMLPEEVEEVIGNKPESDILVHTAYDESTDENVMLLTSDAPEYKPWALVIQDSNGENKIKML

SEQ ID NO: 97 - protein, 1497 aa, synthetic construct
PKKKRKVSSETGPVAVDPTLRRRIEPHEFEVFFDPRELRKETCLLYEINWGGRHSIWRHTSQNTNKHVEVNFIEKFTTERYFCPNTRCSITWFLSWSPCGECSRAITEFLSRYPHVTLFIYIARLYHHADPRNRQGLRDLISSGVTIQIMTEQESGYCWRNFVNYSPSNEAHWPRYPHLWVRLYVLELYCIILGLPPCLNILRRKQPQLTFFTIALQSCHYQRLPPHILWATGLKSGGSSGGSSGSETPGTSESATPESSGGSSGGSMSSAIKSYKSVLRPNERKNQLLKSTIQCLEDGSAFFFKMLQGLFGGITPEIVRFSTEQEKQQQDIALWCAVNWFRPVSQDSLTHTIASDNLVEKFEEYYGGTASDAIKQYFSASIGESYYWNDCRQQYYDLCRELGVEVSDLTHDLEILCREKCLAVATESNQYNSIISVLFGTGRKEDRSVKLRITKKILEAISNLKEIPKNVAPIQEIILNVAKATKETFRQVYAGNLGAPSTLERFIAKDGQKEFDLKKLQTDLKKVIRGKSKERDWCCQEELRSYVEQNTIQYDLWAWGEMFNKAHTALKIKSTRNYNFAKQRLEQFKRIQSLNNLLVVKKLNDFFDSEFFSGEETYTICVHHLGGKRLSKLYKAWEDDPADPENAIVVLCDDLKNNFKKEPIRNILRYIFTIRQECSAQDILAAAKYNQQLDRYKSQKANPSVLGNQGFTWRNAVILPEKAQRNDRPNSLDLRIWLYLKLRHPDGRWKKHHIPFYDTRFFQEIYAAGNSPVDTCQFRTPRFGYHLPKLTDQTAIRVNKKHVKAAKTEARIRLAIQQGTLPVSNLKITRISATINSKGQVRIPVKFDVGRQKGTLQIGDRFCGYDQNQTASHAYSLWEVVKEGQYHKELGCFVRFISSGDIVSITENRGNQFDQLSYEGLAYPQYADWRKKASKFVSLWQITKKNKKKEIVTVEAKEKFDAICKYQPRLYKFNKEYAYLLRDIVRGKSLVELQQIRQEIFRFIEQDCGVTRLGSLSLSTLETVKAVKGIIYSYFSTALNASKNNPISDEQRKEFDPELFALLEKLELIRTRKKKQKVERIANSLIQTCLENNIKFIRGEGDLSTTNNATKKKANSRSMDWLARGVFNKIRQLAPMHNITLFGCGSLYTSHQDPLVHRNPDKAMRARFEEVNVSNVSEWHMRNFSNYLRADSGTGLYYKQATLDFLKHYDLEEHADDLEKQNIKFYDFRKILEDKQLTSVIVPKRGGRIYMATNPVTSDSTPVTYAGKTYNRCNAAHVAAANIALTVKGIGEQSSDEENPDGSRIKLQLTSSGGSGGSGGSTNLSDIIEKETGKQLVIQESILMLPEEVEEVIGNKPESDILVHTAYDESTDENVMLLTSDAPEYKPWALVIQDSNGENKIKMLSGGSGGSGGSTNLSDIIEKETGKQLVIQESILMLPEEVEEVIGNKPESDILVHTAYDESTDENVMLLTSDAPEYKPWALVIQDSNGENKIKML